European Patent Specification EP 3 512 961 B1, published January 10, 2024. Title: INTERNAL AMPLIFICATION CONTROL. Applicant: Qiagen GmbH. The sequence listing filed with the application follows.

SEQUENCE LISTING (4 sequences)

SEQ ID NO: 1 - DNA, 434 bp, Artificial Sequence
  Artificial Sequence
gtagctccataatcagaagatgcgctaccgtacacaacggcggtttaaactttgtagacctcacgcggctgctcaggtcttgcgcatcccatacttcacatggacggaaagctgtgggtttgtatcgataagccgtaggttcctaggatcgagtcacccaaacaacttcgagagctcttctcaccaaccctttgaactccgaaatgccgtgaacacatccccttagttggcattggtctactaaccgagtatcgtacaaagcgagacaggtctggcccctactgcttggatgcgaactaacagtgttcctatatccgtttatactgtggtcgatttcgaaccgatatctcaaagagagcgccggcagagccttagtatcggaactggcgagtgtgtttgggtgaggactattatgtggttggagtagagcgaat

SEQ ID NO: 2 - DNA, 24 bp, Artificial Sequence
  Synthetic Primer
gtagctccataatcagaagatgcg

SEQ ID NO: 3 - DNA, 27 bp, Artificial Sequence
  Synthetic Primer
attcgctctactccaaccacataatag

SEQ ID NO: 4 - DNA, 26 bp, Artificial Sequence
  Synthetic Probe
tccgatactaaggctctgccggcgct